European Patent Application EP 4 548 775 A2, published May 7, 2025. Title: GOLD KIWIFRUIT COMPOSITIONS AND METHODS OF PREPARATION AND USE THEREFOR. Applicant: ANAGENIX IP LIMITED. Application WO PCT/NZ2015/050200, filed November 27, 2015. The sequence listing filed with the application follows.

SEQUENCE LISTING (16 sequences)

SEQ ID NO: 1 - DNA, 50 bp, synthetic construct
  source 1..50: mol_type = other DNA
  misc_feature 46: note = w is a or t
tcgtcggcagcgtcagatgtgtataagagacagcctacgggnggcwgcag

SEQ ID NO: 2 - DNA, 55 bp, synthetic construct
  source 1..55: mol_type = other DNA
  misc_feature 41: note = h is a, c, or t
  misc_feature 42: note = v is a, c, or g
gtctcgtgggctcggagatgtgtataagagacaggactachvgggtatctaatcc

SEQ ID NO: 3 - DNA, 19 bp, synthetic construct
  source 1..19: mol_type = other DNA
tcctacgggaggcagcagt

SEQ ID NO: 4 - DNA, 26 bp, synthetic construct
  source 1..26: mol_type = other DNA
ggactaccagggtatctaatcctgtt

SEQ ID NO: 5 - DNA, 18 bp, synthetic construct
  source 1..18: mol_type = other DNA
gggtggtaatgccggatg

SEQ ID NO: 6 - DNA, 18 bp, synthetic construct
  source 1..18: mol_type = other DNA
ccaccgttacaccgggaa

SEQ ID NO: 7 - DNA, 21 bp, synthetic construct
  source 1..21: mol_type = other DNA
cgatgagtgctaggtgttgga

SEQ ID NO: 8 - DNA, 22 bp, synthetic construct
  source 1..22: mol_type = other DNA
caagatgtcaagacctggtaag

SEQ ID NO: 9 - DNA, 20 bp, synthetic construct
  source 1..20: mol_type = other DNA
ggtgtcggcttaagtgccat

SEQ ID NO: 10 - DNA, 18 bp, synthetic construct
  source 1..18: mol_type = other DNA
cggatgtaagggccgtgc

SEQ ID NO: 11 - DNA, 19 bp, synthetic construct
  source 1..19: mol_type = other DNA
ggaggaagaaggtcttcgg

SEQ ID NO: 12 - DNA, 21 bp, synthetic construct
  source 1..21: mol_type = other DNA
aattccgcctacctctgcact

SEQ ID NO: 13 - DNA, 20 bp, synthetic construct
  source 1..20: mol_type = other DNA
aaatgacggtacctgactaa

SEQ ID NO: 14 - DNA, 22 bp, synthetic construct
  source 1..22: mol_type = other DNA
ctttgagtttcattcttgcgaa

SEQ ID NO: 15 - DNA, 21 bp, synthetic construct
  source 1..21: mol_type = other DNA
gacggtacctgactaagaagc

SEQ ID NO: 16 - DNA, 20 bp, synthetic construct
  source 1..20: mol_type = other DNA
agtttcattcttgcgaacgt